European Patent Application EP 4 682 264 A1, published January 21, 2026. Title: Assay system for the development of antiviral agent for honey bee indicated by inhibition of virus-derived protease. Applicant: Toyama Prefectural University. The sequence listing filed with the application follows.

SEQUENCE LISTING (61 sequences)

SEQ ID NO: 1 - DNA, 26 bp, synthetic construct
  source 1..26: mol_type = other DNA
  misc_feature 1..26: note = probe (ABPV)
atagttaaaacagcttttcacactgg

SEQ ID NO: 2 - DNA, 25 bp, synthetic construct
  source 1..25: mol_type = other DNA
  misc_feature 1..25: note = probe (BQCV)
tttccatctttatcggtacgccgcc

SEQ ID NO: 3 - DNA, 26 bp, synthetic construct
  source 1..26: mol_type = other DNA
  misc_feature 1..26: note = probe (CBPV)
tcaagaacgagaccaccgccaagttc

SEQ ID NO: 4 - DNA, 23 bp, synthetic construct
  source 1..23: mol_type = other DNA
  misc_feature 1..23: note = probe (DWV)
ccttgaccagtagacacagcatc

SEQ ID NO: 5 - DNA, 19 bp, synthetic construct
  source 1..19: mol_type = other DNA
  misc_feature 1..19: note = probe (SBV)
tgatgagagtggacgaaga

SEQ ID NO: 6 - DNA, 30 bp, synthetic construct
  source 1..30: mol_type = other DNA
  misc_feature 1..30: note = probe (VDV-1)
aggtacccatatcaagaataccagttgtcc

SEQ ID NO: 7 - DNA, 24 bp, synthetic construct
  source 1..24: mol_type = other DNA
  misc_feature 1..24: note = probe (IAPV)
tttgcggcaatccagccgtgaaac

SEQ ID NO: 8 - DNA, 19 bp, synthetic construct
  source 1..19: mol_type = other DNA
  misc_feature 1..19: note = probe (KBV)
ctggatggggatattccct

SEQ ID NO: 9 - DNA, 23 bp, synthetic construct
  source 1..23: mol_type = other DNA
  misc_feature 1..23: note = probe (LSV)
tgcggacctcatttcttcatgtc

SEQ ID NO: 10 - DNA, 20 bp, synthetic construct
  source 1..20: mol_type = other DNA
  misc_feature 1..20: note = primer (ABPV)
catattggcgagccactatg

SEQ ID NO: 11 - DNA, 23 bp, synthetic construct
  source 1..23: mol_type = other DNA
  misc_feature 1..23: note = primer (ABPV)
ctaccaggttcaaagaaaatttc

SEQ ID NO: 12 - DNA, 20 bp, synthetic construct
  source 1..20: mol_type = other DNA
  misc_feature 1..20: note = primer (BQCV)
ggtgcgggagatgatatgga

SEQ ID NO: 13 - DNA, 22 bp, synthetic construct
  source 1..22: mol_type = other DNA
  misc_feature 1..22: note = primer (BQCV)
gccgtctgagatgcatgaatac

SEQ ID NO: 14 - DNA, 24 bp, synthetic construct
  source 1..24: mol_type = other DNA
  misc_feature 1..24: note = primer (CBPV)
cgcaagtacgccttgataaagaac

SEQ ID NO: 15 - DNA, 23 bp, synthetic construct
  source 1..23: mol_type = other DNA
  misc_feature 1..23: note = primer (CBPV)
actactagaaactcgtcgcttcg

SEQ ID NO: 16 - DNA, 20 bp, synthetic construct
  source 1..20: mol_type = other DNA
  misc_feature 1..20: note = primer (DWV)
gcggctaagattgtaaattg

SEQ ID NO: 17 - DNA, 22 bp, synthetic construct
  source 1..22: mol_type = other DNA
  misc_feature 1..22: note = primer (DWV)
gtgactagcataaccatgatta

SEQ ID NO: 18 - DNA, 23 bp, synthetic construct
  source 1..23: mol_type = other DNA
  misc_feature 1..23: note = primer (SBV)
aacgtccactacaccgaaatgtc

SEQ ID NO: 19 - DNA, 21 bp, synthetic construct
  source 1..21: mol_type = other DNA
  misc_feature 1..21: note = primer (SBV)
acactgcgcgtctaacattcc

SEQ ID NO: 20 - DNA, 18 bp, synthetic construct
  source 1..18: mol_type = other DNA
  misc_feature 1..18: note = primer (VDV-1)
cgcgtgtcgttcctgatt

SEQ ID NO: 21 - DNA, 24 bp, synthetic construct
  source 1..24: mol_type = other DNA
  misc_feature 1..24: note = primer (VDV-1)
cactcatacgtagtggagcaatta

SEQ ID NO: 22 - DNA, 20 bp, synthetic construct
  source 1..20: mol_type = other DNA
  misc_feature 1..20: note = primer (IAPV)
cgaacttggtgacttgaagg

SEQ ID NO: 23 - DNA, 20 bp, synthetic construct
  source 1..20: mol_type = other DNA
  misc_feature 1..20: note = primer (IAPV)
catcagtcgtcttccaggta

SEQ ID NO: 24 - DNA, 26 bp, synthetic construct
  source 1..26: mol_type = other DNA
  misc_feature 1..26: note = primer (KBV)
atcagaatcaagtgatgccttatcag

SEQ ID NO: 25 - DNA, 26 bp, synthetic construct
  source 1..26: mol_type = other DNA
  misc_feature 1..26: note = primer (KBV)
gcagatggaaatacatctcgcaagtc

SEQ ID NO: 26 - DNA, 21 bp, synthetic construct
  source 1..21: mol_type = other DNA
  misc_feature 1..21: note = primer (LSV)
catcccaagagaaccactyac

SEQ ID NO: 27 - DNA, 20 bp, synthetic construct
  source 1..20: mol_type = other DNA
  misc_feature 1..20: note = primer (LSV)
cgmgtgtgcatggaagagag

SEQ ID NO: 28 - DNA, 500 bp, Acute bee paralysis virus
  source 1..500: mol_type = genomic DNA
atcctgccgtcaaacatgtgctgtcttggaatacaacggataaagttcaagtaccaataagtaatggagatgactggggaggagtgatacctgttggtatgccatgctattctaagataatacggaaaacagagaatgatacaacacaaactaacactgaagttttggatcctgccccttgtgaatatgtttgcaatatgttttcatattggcgagccactatgtgctatcgtatagctatagttaaaacagcttttcacactggcaggttagaaattttctttgaacctggtaggattccgataatgacgacgaaagacaatatttccccggacttgactcaattagatggaaccaaagcgccctccgacaacaattataaatacatcttagatttgactaatgatacggagatcaccataagggtaccttttgtttcaaacaaaatgttcatgaaatctacgggaatttatggtggaaattctgaaaacaattgggat

SEQ ID NO: 29 - DNA, 500 bp, Black queen cell virus
  source 1..500: mol_type = genomic DNA
tgatgtcgcccctactactcatatcagtactcctttggcaatagaacaaatacccataaagggagtcgcagagttccaaataccgtactatgctccatgtttgtcatcttcgtttagagcgaattcggaaacattctactatagttcaggtcggaataatctcgatatagccacatcacctccttccatcaatcgctattatgcggtaggtgcgggagatgatatggacttttccatctttatcggtacgccgccctgtattcatgcatctcagacggctcagtttaccaagataaaacaaggtaaagtgtatgatttgaggtatgatcagtatgaccctttcagggaagtccaggacggtacggcgttcctcaatgctcgtagtattgaggatagcgatttgttgtgagctcctttagagggagggctcactttatctattgcttaaatcggtaagccacaaattttttcaagtgtcatgagtttcttctcggttcttc

SEQ ID NO: 30 - DNA, 500 bp, Chronic bee paralysis virus
  source 1..500: mol_type = genomic DNA
catcaaacgggagtccggatccccgagacactccgttacgccagtgcgtcgaagaattcttaatgacacctcagatgagctggttgaagaaggttcattctcctgtagatttctcgatatgggtcaaacgttaccccgaatggcgccaacggcagctcatcgccgcacgaaatcgcgtcctcagcgacccagaacctcgccgcaagtacgccttgataaagaactttgtcaagaacgagaccaccgccaagttcgtggacccaagaaacatcagtcctcgaagcgacgagtttctagtagtggtgggaccttacatcagcgccatcgaacacgccgcggttcattgcccattcctcatcaaggggctgacaccgaagaagagatgtgataagttatcctggttaacagagtatgagcgatttcttgagatcgacttcgctcgtttcgatcagactctgatgaaagatctcttgcgtattgtcgaattaagatttttactc

SEQ ID NO: 31 - DNA, 500 bp, Deformed wing virus
  source 1..500: mol_type = genomic DNA
cccttgtttaccacaagggttagcgttagacattggttctgctggctctccacatgaaatatttaatagatgtcgtgatggtattataccattaattgcatctggatatagattttatagaggcgatttgcgttataagatcgtttttccaagtaatgttaatagcaacatttgggtacaacatcgaccggatcgtagactggaaggatggtctgcagctaagattgtaaattgtgatgctgtgtctactggtcaaggagtatataatcatggttatgctagtcacattcaaatcacgcgtgtaaataacgttatagaattggaagttccattttataatgctacttgttataattatttacaggcgtttaatgcgtctagcgctgcatctagttatgcagtatctttaggagaaatatcggttggttttcaagctacaagtgatgatattgcatctattgttaacaaacctgttactatttattatagtattggagatg

SEQ ID NO: 32 - DNA, 500 bp, Sacbrood virus
  source 1..500: mol_type = genomic DNA
gtaccaaccgattcctcagttgtggaggaatcagaagaaatcagtcttctgaatatagttcacgcgccagaacctataaaaccaagttggaggcgcgtaatagcggagtggagagattatctacaatccttacctcttgtaagaagacatttgatacagtggactcttataccgatttgtttaatggttgggtttctggtatgtatgttgacaagaacgtccactacaccgaaatgtccagtgatgagagtggacgaagaatctggaatgttagacgcgcagtgtcaattaagaccgcagaaggaactatagtatggcgaaaagttattacctcttacagttgcaaggtggcttcggaactagctgctaagagtatactggtgcaatttgtaggtccaataaggacccagagtgatgaggtaccctcgaaagaatctattcagggggacgctacacagcaaagttccaaggaagaaaatacaataattacacgagaccag

SEQ ID NO: 33 - DNA, 500 bp, Varroa destructor virus-1
  source 1..500: mol_type = genomic DNA
tcgagtgcagattaactcgaataaattccaggttggtcaattacaggcaacttggtactattcggatcatgaaaatttgaatatccagacgaagcgaagtgtgtatggtttttcgcatatggatcatgctttgattagcgcatcagcgagtaatgaagcaaaattagtgataccttttaaacacgtatatccattcttaccaacgcgtgtcgttcctgattggacaactggtattcttgatatgggtaccttaaatattcgtgtaattgctccactacgtatgagtgcgacgggaccaaccacttgtaatgttgtagtatttattaagttaaataatagtgaattcactggcacttcttctggtaagttttacgcgaatcaaatcagggcaaaacctgaaatggaccgtgtgttaaatttggcagaaggattactaaataataccgtaggtggttgtaatatggataatccgtcatatcagcaatctccgcgtcattttg

SEQ ID NO: 34 - DNA, 500 bp, Israeli acute paralysis virus
  source 1..500: mol_type = genomic DNA
gaaattgcaaagcctgtaacaactgctgtaaagtggtttgcagatgttgtcggaactgtggcagctatttttggttggtccaaacctcgaaatcaacaacaggtatgcccattacaaaatgtgcctgcatggggatattctctctataaaggcatagatatgagcgtaccattggcttatgaccctaataacgaacttggtgacttgaaggatgtatttccttctgcggttgatgaaatggctatagggtatgtttgcggcaatccagccgtgaaacatgttcttacctggaagacgactgatgcaattcagaaaccaatagcgaacggagatgattggggtggagttataccagtgggaatgccttgttattctaaatccattagaactacaagtatttcagaaacggaaaatcgtgaaactgaagtcatggatgctgctccatgtgaatatgttgctaacatgttctcatattggcgtgcaactatgtgttataggat

SEQ ID NO: 35 - DNA, 500 bp, Kashmir bee virus
  source 1..500: mol_type = genomic DNA
ttggaccaatttctgaagtggcttcaggggttaagacggctgcaaacggcatcgagcgcattccagtgctaggtgaaattgcaaagccggtaaccgctgcagttaaatggtttgcagacattgtaggaggtgtagcagccatatttgggtggtccaaaccccgaaatcagaatcaagtgatgccttatcagaatgtgcctggatggggatattccctgtacaaaggcattgacatgagcgtgccacttgcttatgaccccaataatgaattaggagacttgcgagatgtatttccatctgctgtagacgaaatggctattgggtatgtttgtggcaatccagctataaaacatgtcctcacctggaatacaacagatgtagtacagaccccaataagtaacggagatgattggggaggagtaataccagtgggaatgccttgctattctaagaccattagatcagttaaaggcgacacttcaactttaaaaaccgaggtg

SEQ ID NO: 36 - DNA, 499 bp, Lake sinai virus
  source 1..499: mol_type = genomic DNA
gactcctctacgtcgggatcagtcttattattcgacgacactgccgaccgagttcatgaggatgactcgtccgcgagatcgacgccgtgtcgaggttctcgattacgtgctaacaagagctacccagggcgcaagtcccgtcgacctgcggaccataactccggcagtgacaaccaaatcgacgttcctcatcccaagagaaccactcaccccctgtgccccgacccgactgcctcgtgcggacctcatttcttcatgtcagtgtgtgagtcaaatgagtcagtacctactctcttccatgcacactcggtgggaggtgaagatatcacccatgttgttgatccggctctgggagcgtctatatcgcaacggtttagcgcttcgcagttacgcctccttggctggtctatcgacggaattttcaatactttatctggcgccgccacctcgtcattcgtcgagtcgacgttgttgtgcttatcacgatttatgcgtgaag

SEQ ID NO: 37 - DNA, 30 bp, synthetic construct
  source 1..30: mol_type = other DNA
  misc_feature 1..30: note = IAPV Cloning primer1-F
cctgtcctatttataccgattttatcgagg

SEQ ID NO: 38 - DNA, 30 bp, synthetic construct
  source 1..30: mol_type = other DNA
  misc_feature 1..30: note = IAPV Cloning primer1-R
attaatgtactatatccagttcaagtgtcg

SEQ ID NO: 39 - DNA, 30 bp, synthetic construct
  source 1..30: mol_type = other DNA
  misc_feature 1..30: note = IAPV Cloning primer2-F
ttagatacgatgaacaacggaaggtttggg

SEQ ID NO: 40 - DNA, 30 bp, synthetic construct
  source 1..30: mol_type = other DNA
  misc_feature 1..30: note = IAPV Cloning primer2-R
tattgtgtacgttgggagtattgctttctt

SEQ ID NO: 41 - DNA, 30 bp, synthetic construct
  source 1..30: mol_type = other DNA
  misc_feature 1..30: note = DWV Cloning primer-F
tttgattcgatatcttggaatactagtgct

SEQ ID NO: 42 - DNA, 30 bp, synthetic construct
  source 1..30: mol_type = other DNA
  misc_feature 1..30: note = DWV Cloning primer-R
ttcatgataagatcgtcgccataacagaca

SEQ ID NO: 43 - DNA, 44 bp, synthetic construct
  source 1..44: mol_type = other DNA
  misc_feature 1..44: note = IAPV T7 primer1-F
taatacgactcactatagggcgaccacccctctcaaacaatctc

SEQ ID NO: 44 - DNA, 44 bp, synthetic construct
  source 1..44: mol_type = other DNA
  misc_feature 1..44: note = IAPV T7 primer1-R
taatacgactcactatagggcgatatatccagttcaagtgtcgg

SEQ ID NO: 45 - DNA, 44 bp, synthetic construct
  source 1..44: mol_type = other DNA
  misc_feature 1..44: note = IAPV T7 primer2-F
taatacgactcactatagggcgagacacaattcttgaaatgcca

SEQ ID NO: 46 - DNA, 44 bp, synthetic construct
  source 1..44: mol_type = other DNA
  misc_feature 1..44: note = IAPV T7 primer2-R
taatacgactcactatagggcgacatgtgttaccatacgactgc

SEQ ID NO: 47 - DNA, 43 bp, synthetic construct
  source 1..43: mol_type = other DNA
  misc_feature 1..43: note = DWV T7 primer-F
taatacgactcactatagggcgacacctggaacatcgggtaag

SEQ ID NO: 48 - DNA, 42 bp, synthetic construct
  source 1..42: mol_type = other DNA
  misc_feature 1..42: note = DWV T7 primer-R
taatacgactcactatagggcgaagagaactcggacaaaggc

SEQ ID NO: 49 - DNA, 40 bp, synthetic construct
  source 1..40: mol_type = other DNA
  misc_feature 1..40: note = GFP T7 primer-F
taatacgactcactatagggacgtaaacggccacaagttc

SEQ ID NO: 50 - DNA, 40 bp, synthetic construct
  source 1..40: mol_type = other DNA
  misc_feature 1..40: note = GFP T7 primer-R
taatacgactcactatagggtgttctgctggtagtggtcg

SEQ ID NO: 51 - protein, 218 aa, Israeli acute paralysis virus
VAQRLITNRVLTNLYKVCLVHNDDRITPLLNGLFVRSNLMLIPGHLLGFIAEYDTIEIRNLFDVVFRVPWKDVKKIPIVNALGESKEAALLAFPKFVCQHSDLVKHFQNAESMSKFKRCEVTLPVLRFSEKVGKFLSTLIECDRVEAYDRPYTLNDSQKGQYILRQGLEYTMPTTNGDCGSPLIINETQVLRKIAGIHVAGATTGKAYAESITQKDLE

SEQ ID NO: 52 - protein, 270 aa, Israeli acute paralysis virus
PNDIVDVTMQMWKDQVAQRLITNRVLTNLYKVCLVHNDDRITPLLNGLFVRSNLMLVPGHLLGFIAEYDTIEIRNLFDVVFRVPWKDVKKILIVNALGESKEAALLAFPKFVCQHSDLVKHFQNAESMSKFKRCEVTLPVLRFSEKVGKFLSTLIECDRVEAYDRPYTLNDSQKGQYILRQGLEYTMPTTNGDCGSPLIINETQVLRKIAGIHVAGATTGKAYAESITQKDLERAFTKIDVSMQIQLDLDSTLDFSKPEPKLPSGTEFGP

SEQ ID NO: 53 - protein, 453 aa, Israeli acute paralysis virus
SSGDCVTRKQQVQRVIEAFASSDAVTLKKSTAKFVESDPNDIVDVTMQMWKDQVAQRLITNRVLTNLYKVCLVHNDDRITPLLNGLFVRSNLMLVPGHLLGFIAEYDTIEIRNLFDVVFRVPWKDVKKIPIVNALGESKEAALLAFPKFVCQHSDLVKHFQNAESMSKFKRCEVTLPVLRFSEKVGKFLSTLIECDRVEAYDRPYTLNDSQKGQYILRQGLEYTMPTTNGDCGSPLIINETQVLRKIAGIHVAGATTGKAYAESITQKDLERAFTKIDVSMQIQLDLDPTLDFSKPEPKLPSGTEFGPEDLSFCDLPALKMLPVGKLSEPLFEPGKTDIRPSLVHGQISDIKTKPAYLRNVIKDGIFVNMKHKNLMKCAMDTPYIDKDMIDEAYQLTKSVWLKGMRDELKKVLTYEEAICGSEVSEYISSINRSSSPGYPWIKDRTKGTKGKQ

SEQ ID NO: 54 - DNA, 657 bp, Israeli acute paralysis virus
  source 1..657: mol_type = genomic DNA
gttgcccaacgattgataaccaaccgtgtgttaacaaacttgtataaggtttgtttagtgcataatgatgaccgcataacacctcttttgaatggactttttgttcgttcaaatttgatgttaattcctggacatcttcttggatttattgctgagtatgatacaatagaaattcgaaatctctttgacgtggtatttagagtaccatggaaagatgtaaagaagattccaattgttaatgctctcggtgaatctaaggaggcagcgttattggcctttccaaaattcgtttgtcaacattctgacttggtcaagcatttccaaaacgctgaatcaatgtctaaattcaaacgttgtgaagtaaccctcccagtattacgtttctctgagaaagttggtaaatttttatcaacactcatagaatgcgatcgggtggaggcttatgacagaccatatacgctgaatgactctcaaaaaggacaatatattctacgtcaaggcttagaatatacgatgccaacgaccaatggtgattgtggttcgccactaatcatcaatgaaacccaagttttgaggaaaattgctggtattcatgtggcaggagctacaactggtaaggcctatgctgaatctataacccaaaaagatcttgagtaa

SEQ ID NO: 55 - DNA, 813 bp, Israeli acute paralysis virus
  source 1..813: mol_type = genomic DNA
ccaaatgacatagttgatgttacaatgcaaatgtggaaggatcaagttgctcaacgactgataactaaccgtgtgttaacaaacttgtataaggtttgtttagtgcataatgacgatcgcattacacctcttttgaatggactttttgttcgttcgaatttgatgttagttcctggacatcttcttggatttattgctgagtatgatacaatagaaattcgaaatctctttgacgtggtatttagagtaccatggaaagatgtaaagaagattctaattgttaatgctctcggtgaatctaaggaggcagcgttattggcctttccaaaattcgtttgtcaacattctgacttggtcaagcatttccaaaatgctgaatcaatgtctaaattcaaacgatgtgaagtaaccctcccagtattacgtttctctgagaaagttggtaaatttttatcaacactcatagaatgcgatcgggtggaggcttatgacagaccatatacgctgaatgactctcaaaaaggacaatatattctacgtcaaggcttagaatatacgatgccaacgaccaatggtgattgtggttcgccactaatcatcaacgaaacccaagttttgaggaaaattgctggtattcatgtggcaggagctacaaccggtaaggcctatgctgaatctataacccaaaaagatcttgagcgagcatttactaaaatagatgtgagcatgcagatccaattggatttggattcgacattggacttctcaaaacctgaacctaaattgccttctggtactgaatttggtccttaa

SEQ ID NO: 56 - DNA, 1362 bp, Israeli acute paralysis virus
  source 1..1362: mol_type = genomic DNA
tcttctggtgattgtgtgacccgaaaacaacaagtgcaacgagtgattgaagcatttgcaagtagtgatgctgtgacattaaagaaatctactgcgaaattcgtagaaagtgacccaaatgacatagttgatgttacaatgcaaatgtggaaggatcaagttgctcaacgactgataactaaccgtgtgttaacaaacttgtataaggtttgtttagtgcataatgacgatcgcattacacctcttttgaatggactttttgttcgttcaaatttgatgttagttcctggacatcttcttggatttattgctgagtatgatacaatagaaattcgaaatctctttgacgtggtatttagagtaccatggaaagatgtaaagaagattccaattgttaatgctctcggtgaatctaaggaggcagcgttattggcctttccaaaattcgtttgtcaacattctgacttggtcaagcatttccaaaacgctgaatcaatgtctaaattcaaacgttgtgaagtaaccctcccagtattacgtttctctgagaaagttggtaaatttttatcaacactcatagaatgcgatcgggtggaggcttatgacagaccatatacgctgaatgactctcaaaaaggacaatatattctacgtcaaggcttagaatatacgatgccaacgaccaatggtgattgtggttcgccactaatcatcaacgaaacccaagttttgaggaaaattgctggtattcatgtggcaggagctacaaccggtaaggcctatgctgaatctataacccaaaaagatcttgagcgagcatttactaaaatagacgtgagcatgcagatccaattggatttggatccgacattggacttctcaaaacctgaacctaaattgccttctggtactgaatttggtcctgaagatctcagcttctgtgatcttccggccctaaagatgttaccagtaggtaaactttccgaacccttatttgaacctggcaaaacagatataaggccttccttggtacatggtcagattagcgacataaaaacaaaacccgcctacttacgtaatgtgattaaagatggaatttttgttaatatgaaacataagaatctgatgaaatgtgctatggatacaccttatatcgacaaggacatgattgatgaggcataccagttaaccaaatctgtttggttaaaaggtatgagagatgaattgaagaaggttctcacttatgaagaagccatttgtggctctgaagtaagtgagtatatttcttcaataaatcggagtagttcccctggatatccttggattaaggacagaacaaaaggaactaaaggaaaacaataa

SEQ ID NO: 57 - DNA, 675 bp, Israeli acute paralysis virus
  source 1..675: mol_type = genomic DNA
gttgctcaacgactgataactaaccgtgtgttaacaaacttgtataaggtttgtttagtgcataatgacgatcgcattacacctcttttgaatggactttttgttcgttcgaatttgatgttagttcctggacatcttcttggatttattgctgagtatgatacaatagaaattcgaaatctctttgacgtggtatttagagtaccatggaaagatgtaaagaagattctaattgttaatgctctcggtgaatctaaggaggcagcgttattggcctttccaaaattcgtttgtcaacattctgacttggtcaagcatttccaaaatgctgaatcaatgtctaaattcaaacgatgtgaagtaaccctcccagtattacgtttctctgagaaagttggtaaatttttatcaacactcatagaatgcgatcgggtggaggcttatgacagaccatatacgctgaatgactctcaaaaaggacaatatattctacgtcaaggcttagaatatacgatgccaacgaccaatggtgattgtggttcgccactaatcatcaacgaaacccaagttttgaggaaaattgctggtattcatgtggcaggagctacaaccggtaaggcctatgctgaatctataacccaaaaagatcttgagcgagcatttactaaaatataa

SEQ ID NO: 58 - protein, 224 aa, Israeli acute paralysis virus
VAQRLITNRVLTNLYKVCLVHNDDRITPLLNGLFVRSNLMLVPGHLLGFIAEYDTIEIRNLFDVVFRVPWKDVKKILIVNALGESKEAALLAFPKFVCQHSDLVKHFQNAESMSKFKRCEVTLPVLRFSEKVGKFLSTLIECDRVEAYDRPYTLNDSQKGQYILRQGLEYTMPTTNGDCGSPLIINETQVLRKIAGIHVAGATTGKAYAESITQKDLERAFTKI

SEQ ID NO: 59 - DNA, 39 bp, synthetic construct
  source 1..39: mol_type = other DNA
  misc_feature 1..39: note = IAPV Protease Primer-F1
cgcggatccccaaatgacatagttgatgttacaatgcaa

SEQ ID NO: 60 - DNA, 33 bp, synthetic construct
  source 1..33: mol_type = other DNA
  misc_feature 1..33: note = IAPV Protease Primer-R
cccaagcttttatattttagtaaatgctcgctc

SEQ ID NO: 61 - DNA, 39 bp, synthetic construct
  source 1..39: mol_type = other DNA
  misc_feature 1..39: note = IAPV Protease Primer-F2
cgcggatccgttgcccaacgattgataaccaaccgtgta